European Patent Application EP 4 130 269 A1, published February 8, 2023. Title: Antibody that binds to fibrin and composition comprising the same. Applicant: National Cancer Center Japan Rin Institute Inc. The sequence listing filed with the application follows.

SEQUENCE LISTING (18 sequences)

SEQ ID NO: 1 - protein, 5 aa, Artificial Sequence
  HCDR1 of humanized 1101 clone
SYWMH

SEQ ID NO: 2 - protein, 17 aa, Artificial Sequence
  HCDR2 of humanized 1101 clone
AIYPGNSDTRYSPSFQG

SEQ ID NO: 3 - protein, 11 aa, Artificial Sequence
  HCDR3 of humanized 1101 clone
KAHYGNYGFAY

SEQ ID NO: 4 - protein, 11 aa, Artificial Sequence
  LCDR1 of humanized 1101 clone
RASQHINNWLA

SEQ ID NO: 5 - protein, 7 aa, Artificial Sequence
  LCDR2 of humanized 1101 clone
GATSLQS

SEQ ID NO: 6 - protein, 9 aa, Artificial Sequence
  LCDR3 of humanized 1101 clone
QQYWSTPLT

SEQ ID NO: 7 - protein, 242 aa, Artificial Sequence
  Fab region of heavy chain of humanized 1101 clone
MGSTAILALLLAVLQGVCAEVQLVQSGAEVKKPGESLKISCKGSGYSFTSYWMHWVRQMPGKGLEWIGAIYPGNSDTRYSPSFQGQVTISADKSISTAYLQWSSLKASDTAMYYCTRKAHYGNYGFAYWGQGTLVTVSSASTKGPSVFPLAPSSKSTSGGTAALGCLVKDYFPEPVTVSWNSGALTSGVHTFPAVLQSSGLYSLSSVVTVPSSSLGTQTYICNVNHKPSNTKVDKKVEPKSC

SEQ ID NO: 8 - protein, 236 aa, Artificial Sequence
  Light chain of humanized 1101 clone
MDMRVPAQLLGLLLLWLRGARCDIQMTQSPSSLSASVGDRVTITCRASQHINNWLAWYQQKPGKAPKLLISGATSLQSGVPSRFSGSGSGTDFTLTISSLQPEDFATYYCQQYWSTPLTFGQGTKVEIKRTVAAPSVFIFPPSDEQLKSGTASVVCLLNNFYPREAKVQWKVDNALQSGNSQESVTEQDSKDSTYSLSSTLTLSKADYEKHKVYACEVTHQGLSSPVTKSFNRGEC

SEQ ID NO: 9 - protein, 5 aa, Artificial Sequence
  HCDR1 of humanized 99 antibody
NYGMN

SEQ ID NO: 10 - protein, 17 aa, Artificial Sequence
  HCDR2 of humanized 99 antibody
WINTKIGEPTYAQKFQG

SEQ ID NO: 11 - protein, 4 aa, Artificial Sequence
  HCDR3 of humanized 99 antibody
LLDY

SEQ ID NO: 12 - protein, 17 aa, Artificial Sequence
  LCDR1 of humanized 99 antibody
RASQSVLYSSNQKNYLA

SEQ ID NO: 13 - protein, 7 aa, Artificial Sequence
  LCDR2 of humanized 99 antibody
WASSLQS

SEQ ID NO: 14 - protein, 8 aa, Artificial Sequence
  LCDR3 of humanized 99 antibody
HQYLSSYT

SEQ ID NO: 15 - protein, 113 aa, Artificial Sequence
  Heavy chain variable region of humanized 99 antibody
QVQLVQSGAEVKKPGASVKVSCKASGYTFTNYGMNWVRQAPGQGLEWMGWINTKIGEPTYAQKFQGRVTMTRDKSSSTAYMELSSLRSEDTAVYYCARLLDYWGQGTLVTVSS

SEQ ID NO: 16 - protein, 113 aa, Artificial Sequence
  Light chain varible region of humanized 99 antibody
DIQMTQSPSSLSASVGDRVTITCRASQSVLYSSNQKNYLAWYQQKPGKSPKLLIYWASSLQSGVPSRFSGSGSGTDFTLTISSLQPEDFATYYCHQYLSSYTFGQGTKVEIKR

SEQ ID NO: 17 - protein, 16 aa, Artificial Sequence
  Fibrinogen Bbeta 231-246
CNIPVVSGKECEEIIR

SEQ ID NO: 18 - protein, 15 aa, Artificial Sequence
  Fibrinogen gamma 232-246
KNWIQYKEGFGHLSP